European Patent Specification EP 3 642 344 B1, published December 4, 2024. Title: METHODS AND COMPOSITIONS FOR CHIMERIC ANTIGEN RECEPTOR TARGETING CANCER CELLS. Applicant: The University of North Carolina at Chapel Hill The General Hospital Corporation Dotti, Gianpietro Ferrone, Soldano Du, Hongwei Wang, Xinhui Ferrone, Cristina. The sequence listing filed with the application follows.

SEQUENCE LISTING (5 sequences)

SEQ ID NO: 1 - protein, 483 aa, Artificial
  chimeric antigen receptor CD28
MEFGLSWLFLVAILKGVQCDIVMTQSHKFMSTSIGARVSITCKASQDVRTAVAWYQQKPGQSPKLLIYSASYRYTGVPDRFTGSGSGTDFTFTISSVQAEDLAVYYCQQHYGTPPWTFGGGTKLEIKGGGGSGGGGSGGGGSEVQLVESGGGLVKPGGSLKLSCEASRFTFSSYAMSWVRQTPEKRLEWVAAISGGGRYTYYPDSMKGRFTISRDNAKNFLYLQMSSLRSEDTAMYYCARHYDGYLDYWGQGTTLTVSSTRTTTPAPRPPTPAPTIASQPLSLRPEACRPAAGGAVHTRGLDFACDIYIWAPLAGTCGVLLLSLVITLYCRSKRSRLLHSDYMNMTPRRPGPTRKHYQPYAPPRDFAAYRSRVKFSRSADAPAYQQGQNQLYNELNLGRREEYDVLDKRRGRDPEMGGKPRRKNPQEGLYNELQKDKMAEAYSEIGMKGERRRGKGHDGLYQGLSTATKDTYDALHMQALPPR

SEQ ID NO: 2 - protein, 484 aa, Artificial
  chimeric antigen receptor 4-1-BB
MEFGLSWLFLVAILKGVQCDIVMTQSHKFMSTSIGARVSITCKASQDVRTAVAWYQQKPGQSPKLLIYSASYRYTGVPDRFTGSGSGTDFTFTISSVQAEDLAVYYCQQHYGTPPWTFGGGTKLEIKGGGGSGGGGSGGGGSEVQLVESGGGLVKPGGSLKLSCEASRFTFSSYAMSWVRQTPEKRLEWVAAISGGGRYTYYPDSMKGRFTISRDNAKNFLYLQMSSLRSEDTAMYYCARHYDGYLDYWGQGTTLTVSSTRTTTPAPRPPTPAPTIASQPLSLRPEACRPAAGGAVHTRGLDFACDIYIWAPLAGTCGVLLLSLVITLYCKRGRKKLLYIFKQPFMRPVQTTQEEDGCSCRFPEEEEGGCELRVKFSRSADAPAYQQGQNQLYNELNLGRREEYDVLDKRRGRDPEMGGKPRRKNPQEGLYNELQKDKMAEAYSEIGMKGERRRGKGHDGLYQGLSTATKDTYDALHMQALPPR

SEQ ID NO: 3 - DNA, 7811 bp, Artificial
  plasmid CD28
aagctttgctcttaggagtttcctaatacatcccaaactcaaatatataaagcatttgacttgttctatgccctagggggcggggggaagctaagccagctttttttaacatttaaaatgttaattccattttaaatgcacagatgtttttatttcataagggtttcaatgtgcatgaatgctgcaatattcctgttaccaaagctagtataaataaaaatagataaacgtggaaattacttagagtttctgtcattaacgtttccttcctcagttgacaacataaatgcgctgctgagcaagccagtttgcatctgtcaggatcaatttcccattatgccagtcatattaattactagtcaattagttgatttttatttttgacatatacatgtgaatgaaagaccccacctgtaggtttggcaagctagcttaagtaacgccattttgcaaggcatggaaaaatacataactgagaatagaaaagttcagatcaaggtcaggaacagatggaacagctgaatatgggccaaacaggatatctgtggtaagcagttcctgccccggctcagggccaagaacagatggaacagctgaatatgggccaaacaggatatctgtggtaagcagttcctgccccggctcagggccaagaacagatggtccccagatgcggtccagccctcagcagtttctagagaaccatcagatgtttccagggtgccccaaggacctgaaatgaccctgtgccttatttgaactaaccaatcagttcgcttctcgcttctgttcgcgcgcttatgctccccgagctcaataaaagagcccacaacccctcactcggggcgccagtcctccgattgactgagtcgcccgggtacccgtgtatccaataaaccctcttgcagttgcatccgacttgtggtctcgctgttccttgggagggtctcctctgagtgattgactacccgtcagcgggggtctttcatttgggggctcgtccgggatcgggagacccctgcccagggaccaccgacccaccaccgggaggtaagctggccagcaacttatctgtgtctgtccgattgtctagtgtctatgactgattttatgcgcctgcgtcggtactagttagctaactagctctgtatctggcggacccgtggtggaactgacgagttcggaacacccggccgcaaccctgggagacgtcccagggacttcgggggccgtttttgtggcccgacctgagtcctaaaatcccgatcgtttaggactctttggtgcaccccccttagaggagggatatgtggttctggtaggagacgagaacctaaaacagttcccgcctccgtctgaatttttgctttcggtttgggaccgaagccgcgccgcgcgtcttgtctgctgcagcatcgttctgtgttgtctctgtctgactgtgtttctgtatttgtctgaaaatatgggcccgggctagcctgttaccactcccttaagtttgaccttaggtcactggaaagatgtcgagcggatcgctcacaaccagtcggtagatgtcaagaagagacgttgggttaccttctgctctgcagaatggccaacctttaacgtcggatggccgcgagacggcacctttaaccgagacctcatcacccaggttaagatcaaggtcttttcacctggcccgcatggacacccagaccaggtggggtacatcgtgacctgggaagccttggcttttgacccccctccctgggtcaagccctttgtacaccctaagcctccgcctcctcttcctccatccgccccgtctctcccccttgaacctcctcgttcgaccccgcctcgatcctccctttatccagccctcactccttctctaggcgcccccatatggccatatgagatcttatatggggcacccccgccccttgtaaacttccctgaccctgacatgacaagagttactaacagcccctctctccaagctcacttacaggctctctacttagtccagcacgaagtctggagacctctggcggcagcctaccaagaacaactggaccgaccggtggtacctcacccttaccgagtcggcgacacagtgtgggtccgccgacaccagactaagaacctagaacctcgctggaaaggaccttacacagtcctgctgaccacccccaccgccctcaaagtagacggcatcgcagcttggatacacgccgcccacgtgaaggctgccgaccccgggggtggaccatcctctagactgccatggaattcggcctgagctggctgttcctggtggccatcctgaagggcgtgcagtgcgacattgtgatgacccagtctcacaaattcatgtccacatcaattggagccagggtcagcatcacctgcaaggccagtcaggatgtgagaactgctgtagcctggtatcaacagaaaccaggccagtctcctaaactactaatttactcggcatcctaccggtacactggagtccctgatcgcttcactggcagtggatctgggacggatttcactttcaccatcagcagtgtgcaggctgaagacctggcagtttattactgtcagcaacattatggtactcctccgtggacgttcggtggaggcaccaagctggaaatcaaaggcggcggaggatctggcggaggcggaagtggcggagggggctctgaagtgcagctggtggagtctgggggaggcttagtgaagcctggagggtccctgaaactctcctgtgaagcctctagattcactttcagtagctatgccatgtcttgggttcgccagactccggagaagaggctggagtgggtcgcagccattagtggaggtggtaggtacacctactatccagacagtatgaagggtcgattcaccatctccagagacaatgccaagaatttcctgtacctgcaaatgagcagtctgaggtctgaggacacggccatgtattactgtgcaagacactatgatggttatcttgactactggggccaaggcaccactctcacagtctcctcaacgcgtaccacgacgccagcgccgcgaccaccaacaccggcgcccaccatcgcgtcgcagcccctgtccctgcgcccagaggcgtgccggccagcggcggggggcgcagtgcacacgagggggctggacttcgcctgtgatatctacatctgggcgcccttggccgggacttgtggggtccttctcctgtcactggttatcaccctttactgcaggagtaagaggagcaggctcctgcacagtgactacatgaacatgactccccgccgccccgggcccacccgcaagcattaccagccctatgccccaccacgcgacttcgcagcctatcgctccagagtgaagttcagcaggagcgcagacgcccccgcgtaccagcagggccagaaccagctctataacgagctcaatctaggacgaagagaggagtacgatgttttggacaagagacgtggccgggaccctgagatggggggaaagccgagaaggaagaaccctcaggaaggcctgtacaatgaactgcagaaagataagatggcggaggcctacagtgagattgggatgaaaggcgagcgccggaggggcaaggggcacgatggcctttaccagggtctcagtacagccaccaaggacacctacgacgcccttcacatgcaggccctgccccctcgctaagcatgcacctcgagatcgatccggattagtccaatttgttaaagacaggatatcagtggtccaggctctagttttgactcaacaatatcaccagctgaagcctatagagtacgagccatagataaaataaaagattttatttagtctccagaaaaaggggggaatgaaagaccccacctgtaggtttggcaagctagcttaagtaacgccattttgcaaggcatggaaaaatacataactgagaatagagaagttcagatcaaggtcaggaacagatggaacagctgaatatgggccaaacaggatatctgtggtaagcagttcctgccccggctcagggccaagaacagatggaacagctgaatatgggccaaacaggatatctgtggtaagcagttcctgccccggctcagggccaagaacagatggtccccagatgcggtccagccctcagcagtttctagagaaccatcagatgtttccagggtgccccaaggacctgaaatgaccctgtgccttatttgaactaaccaatcagttcgcttctcgcttctgttcgcgcgcttctgctccccgagctcaataaaagagcccacaacccctcactcggggcgccagtcctccgattgactgagtcgcccgggtacccgtgtatccaataaaccctcttgcagttgcatccgacttgtggtctcgctgttccttgggagggtctcctctgagtgattgactacccgtcagcgggggtctttcacacatgcagcatgtatcaaaattaatttggttttttttcttaagtatttacattaaatggccatagtacttaaagttacattggcttccttgaaataaacatggagtattcagaatgtgtcataaatatttctaattttaagatagtatctccattggctttctactttttcttttatttttttttgtcctctgtcttccatttgttgttgttgttgtttgtttgtttgtttgttggttggttggttaatttttttttaaagatcctacactatagttcaagctagactattagctactctgtaacccagggtgaccttgaagtcatgggtagcctgctgttttagccttcccacatctaagattacaggtatgagctatcatttttggtatattgattgattgattgattgatgtgtgtgtgtgtgattgtgtttgtgtgtgtgactgtgaaaatgtgtgtatgggtgtgtgtgaatgtgtgtatgtatgtgtgtgtgtgagtgtgtgtgtgtgtgtgtgcatgtgtgtgtgtgtgactgtgtctatgtgtatgactgtgtgtgtgtgtgtgtgtgtgtgtgtgtgtgtgtgtgtgtgtgtgttgtgaaaaaatattctatggtagtgagagccaacgctccggctcaggtgtcaggttggtttttgagacagagtctttcacttagcttggaattcactggccgtcgttttacaacgtcgtgactgggaaaaccctggcgttacccaacttaatcgccttgcagcacatccccctttcgccagctggcgtaatagcgaagaggcccgcaccgatcgcccttcccaacagttgcgcagcctgaatggcgaatggcgcctgatgcggtattttctccttacgcatctgtgcggtatttcacaccgcatatggtgcactctcagtacaatctgctctgatgccgcatagttaagccagccccgacacccgccaacacccgctgacgcgccctgacgggcttgtctgctcccggcatccgcttacagacaagctgtgaccgtctccgggagctgcatgtgtcagaggttttcaccgtcatcaccgaaacgcgcgatgacgaaagggcctcgtgatacgcctatttttataggttaatgtcatgataataatggtttcttagacgtcaggtggcacttttcggggaaatgtgcgcggaacccctatttgtttatttttctaaatacattcaaatatgtatccgctcatgagacaataaccctgataaatgcttcaataatattgaaaaaggaagagtatgagtattcaacatttccgtgtcgcccttattcccttttttgcggcattttgccttcctgtttttgctcacccagaaacgctggtgaaagtaaaagatgctgaagatcagttgggtgcacgagtgggttacatcgaactggatctcaacagcggtaagatccttgagagttttcgccccgaagaacgttttccaatgatgagcacttttaaagttctgctatgtggcgcggtattatcccgtattgacgccgggcaagagcaactcggtcgccgcatacactattctcagaatgacttggttgagtactcaccagtcacagaaaagcatcttacggatggcatgacagtaagagaattatgcagtgctgccataaccatgagtgataacactgcggccaacttacttctgacaacgatcggaggaccgaaggagctaaccgcttttttgcacaacatgggggatcatgtaactcgccttgatcgttgggaaccggagctgaatgaagccataccaaacgacgagcgtgacaccacgatgcctgtagcaatggcaacaacgttgcgcaaactattaactggcgaactacttactctagcttcccggcaacaattaatagactggatggaggcggataaagttgcaggaccacttctgcgctcggcccttccggctggctggtttattgctgataaatctggagccggtgagcgtgggtctcgcggtatcattgcagcactggggccagatggtaagccctcccgtatcgtagttatctacacgacggggagtcaggcaactatggatgaacgaaatagacagatcgctgagataggtgcctcactgattaagcattggtaactgtcagaccaagtttactcatatatactttagattgatttaaaacttcatttttaatttaaaaggatctaggtgaagatcctttttgataatctcatgaccaaaatcccttaacgtgagttttcgttccactgagcgtcagaccccgtagaaaagatcaaaggatcttcttgagatcctttttttctgcgcgtaatctgctgcttgcaaacaaaaaaaccaccgctaccagcggtggtttgtttgccggatcaagagctaccaactctttttccgaaggtaactggcttcagcagagcgcagataccaaatactgtccttctagtgtagccgtagttaggccaccacttcaagaactctgtagcaccgcctacatacctcgctctgctaatcctgttaccagtggctgctgccagtggcgataagtcgtgtcttaccgggttggactcaagacgatagttaccggataaggcgcagcggtcgggctgaacggggggttcgtgcacacagcccagcttggagcgaacgacctacaccgaactgagatacctacagcgtgagcattgagaaagcgccacgcttcccgaagggagaaaggcggacaggtatccggtaagcggcagggtcggaacaggagagcgcacgagggagcttccagggggaaacgcctggtatctttatagtcctgtcgggtttcgccacctctgacttgagcgtcgatttttgtgatgctcgtcaggggggcggagcctatggaaaaacgccagcaacgcggcctttttacggttcctggccttttgctggccttttgctcacatgttctttcctgcgttatcccctgattctgtggataaccgtattaccgcctttgagtgagctgataccgctcgccgcagccgaacgaccgagcgcagcgagtcagtgagcgaggaagcggaagagcgcccaatacgcaaaccgcctctccccgcgcgttggccgattcattaatgcagctggcacgacaggtttcccgactggaaagcgggcagtgagcgcaacgcaattaatgtgagttagctcactcattaggcaccccaggctttacactttatgcttccggctcgtatgttgtgtggaattgtgagcggataacaatttcacacaggaaacagctatgaccatgattacgcc

SEQ ID NO: 4 - DNA, 7814 bp, Artificial
  plasmid 4-1-BB
aagctttgctcttaggagtttcctaatacatcccaaactcaaatatataaagcatttgacttgttctatgccctagggggcggggggaagctaagccagctttttttaacatttaaaatgttaattccattttaaatgcacagatgtttttatttcataagggtttcaatgtgcatgaatgctgcaatattcctgttaccaaagctagtataaataaaaatagataaacgtggaaattacttagagtttctgtcattaacgtttccttcctcagttgacaacataaatgcgctgctgagcaagccagtttgcatctgtcaggatcaatttcccattatgccagtcatattaattactagtcaattagttgatttttatttttgacatatacatgtgaatgaaagaccccacctgtaggtttggcaagctagcttaagtaacgccattttgcaaggcatggaaaaatacataactgagaatagaaaagttcagatcaaggtcaggaacagatggaacagctgaatatgggccaaacaggatatctgtggtaagcagttcctgccccggctcagggccaagaacagatggaacagctgaatatgggccaaacaggatatctgtggtaagcagttcctgccccggctcagggccaagaacagatggtccccagatgcggtccagccctcagcagtttctagagaaccatcagatgtttccagggtgccccaaggacctgaaatgaccctgtgccttatttgaactaaccaatcagttcgcttctcgcttctgttcgcgcgcttatgctccccgagctcaataaaagagcccacaacccctcactcggggcgccagtcctccgattgactgagtcgcccgggtacccgtgtatccaataaaccctcttgcagttgcatccgacttgtggtctcgctgttccttgggagggtctcctctgagtgattgactacccgtcagcgggggtctttcatttgggggctcgtccgggatcgggagacccctgcccagggaccaccgacccaccaccgggaggtaagctggccagcaacttatctgtgtctgtccgattgtctagtgtctatgactgattttatgcgcctgcgtcggtactagttagctaactagctctgtatctggcggacccgtggtggaactgacgagttcggaacacccggccgcaaccctgggagacgtcccagggacttcgggggccgtttttgtggcccgacctgagtcctaaaatcccgatcgtttaggactctttggtgcaccccccttagaggagggatatgtggttctggtaggagacgagaacctaaaacagttcccgcctccgtctgaatttttgctttcggtttgggaccgaagccgcgccgcgcgtcttgtctgctgcagcatcgttctgtgttgtctctgtctgactgtgtttctgtatttgtctgaaaatatgggcccgggctagcctgttaccactcccttaagtttgaccttaggtcactggaaagatgtcgagcggatcgctcacaaccagtcggtagatgtcaagaagagacgttgggttaccttctgctctgcagaatggccaacctttaacgtcggatggccgcgagacggcacctttaaccgagacctcatcacccaggttaagatcaaggtcttttcacctggcccgcatggacacccagaccaggtggggtacatcgtgacctgggaagccttggcttttgacccccctccctgggtcaagccctttgtacaccctaagcctccgcctcctcttcctccatccgccccgtctctcccccttgaacctcctcgttcgaccccgcctcgatcctccctttatccagccctcactccttctctaggcgcccccatatggccatatgagatcttatatggggcacccccgccccttgtaaacttccctgaccctgacatgacaagagttactaacagcccctctctccaagctcacttacaggctctctacttagtccagcacgaagtctggagacctctggcggcagcctaccaagaacaactggaccgaccggtggtacctcacccttaccgagtcggcgacacagtgtgggtccgccgacaccagactaagaacctagaacctcgctggaaaggaccttacacagtcctgctgaccacccccaccgccctcaaagtagacggcatcgcagcttggatacacgccgcccacgtgaaggctgccgaccccgggggtggaccatcctctagactgccatggaattcggcctgagctggctgttcctggtggccatcctgaagggcgtgcagtgcgacattgtgatgacccagtctcacaaattcatgtccacatcaattggagccagggtcagcatcacctgcaaggccagtcaggatgtgagaactgctgtagcctggtatcaacagaaaccaggccagtctcctaaactactaatttactcggcatcctaccggtacactggagtccctgatcgcttcactggcagtggatctgggacggatttcactttcaccatcagcagtgtgcaggctgaagacctggcagtttattactgtcagcaacattatggtactcctccgtggacgttcggtggaggcaccaagctggaaatcaaaggcggcggaggatctggcggaggcggaagtggcggagggggctctgaagtgcagctggtggagtctgggggaggcttagtgaagcctggagggtccctgaaactctcctgtgaagcctctagattcactttcagtagctatgccatgtcttgggttcgccagactccggagaagaggctggagtgggtcgcagccattagtggaggtggtaggtacacctactatccagacagtatgaagggtcgattcaccatctccagagacaatgccaagaatttcctgtacctgcaaatgagcagtctgaggtctgaggacacggccatgtattactgtgcaagacactatgatggttatcttgactactggggccaaggcaccactctcacagtctcctcaacgcgtaccacgacgccagcgccgcgaccaccaacaccggcgcccaccatcgcgtcgcagcccctgtccctgcgcccagaggcgtgccggccagcggcggggggcgcagtgcacacgagggggctggacttcgcctgtgatatctacatctgggcgcccttggccgggacttgtggggtccttctcctgtcactggttatcaccctttactgcaaacggggcagaaagaaactcctgtatatattcaaacaaccatttatgagaccagtacaaactactcaagaggaagatggctgtagctgccgatttccagaagaagaagaaggaggatgtgaactgagagtgaagttcagcaggagcgcagacgcccccgcgtaccagcagggccagaaccagctctataacgagctcaatctaggacgaagagaggagtacgatgttttggacaagagacgtggccgggaccctgagatggggggaaagccgagaaggaagaaccctcaggaaggcctgtacaatgaactgcagaaagataagatggcggaggcctacagtgagattgggatgaaaggcgagcgccggaggggcaaggggcacgatggcctttaccagggtctcagtacagccaccaaggacacctacgacgcccttcacatgcaggccctgccccctcgctaagcatgcacctcgagatcgatccggattagtccaatttgttaaagacaggatatcagtggtccaggctctagttttgactcaacaatatcaccagctgaagcctatagagtacgagccatagataaaataaaagattttatttagtctccagaaaaaggggggaatgaaagaccccacctgtaggtttggcaagctagcttaagtaacgccattttgcaaggcatggaaaaatacataactgagaatagagaagttcagatcaaggtcaggaacagatggaacagctgaatatgggccaaacaggatatctgtggtaagcagttcctgccccggctcagggccaagaacagatggaacagctgaatatgggccaaacaggatatctgtggtaagcagttcctgccccggctcagggccaagaacagatggtccccagatgcggtccagccctcagcagtttctagagaaccatcagatgtttccagggtgccccaaggacctgaaatgaccctgtgccttatttgaactaaccaatcagttcgcttctcgcttctgttcgcgcgcttctgctccccgagctcaataaaagagcccacaacccctcactcggggcgccagtcctccgattgactgagtcgcccgggtacccgtgtatccaataaaccctcttgcagttgcatccgacttgtggtctcgctgttccttgggagggtctcctctgagtgattgactacccgtcagcgggggtctttcacacatgcagcatgtatcaaaattaatttggttttttttcttaagtatttacattaaatggccatagtacttaaagttacattggcttccttgaaataaacatggagtattcagaatgtgtcataaatatttctaattttaagatagtatctccattggctttctactttttcttttatttttttttgtcctctgtcttccatttgttgttgttgttgtttgtttgtttgtttgttggttggttggttaatttttttttaaagatcctacactatagttcaagctagactattagctactctgtaacccagggtgaccttgaagtcatgggtagcctgctgttttagccttcccacatctaagattacaggtatgagctatcatttttggtatattgattgattgattgattgatgtgtgtgtgtgtgattgtgtttgtgtgtgtgactgtgaaaatgtgtgtatgggtgtgtgtgaatgtgtgtatgtatgtgtgtgtgtgagtgtgtgtgtgtgtgtgtgcatgtgtgtgtgtgtgactgtgtctatgtgtatgactgtgtgtgtgtgtgtgtgtgtgtgtgtgtgtgtgtgtgtgtgtgtgttgtgaaaaaatattctatggtagtgagagccaacgctccggctcaggtgtcaggttggtttttgagacagagtctttcacttagcttggaattcactggccgtcgttttacaacgtcgtgactgggaaaaccctggcgttacccaacttaatcgccttgcagcacatccccctttcgccagctggcgtaatagcgaagaggcccgcaccgatcgcccttcccaacagttgcgcagcctgaatggcgaatggcgcctgatgcggtattttctccttacgcatctgtgcggtatttcacaccgcatatggtgcactctcagtacaatctgctctgatgccgcatagttaagccagccccgacacccgccaacacccgctgacgcgccctgacgggcttgtctgctcccggcatccgcttacagacaagctgtgaccgtctccgggagctgcatgtgtcagaggttttcaccgtcatcaccgaaacgcgcgatgacgaaagggcctcgtgatacgcctatttttataggttaatgtcatgataataatggtttcttagacgtcaggtggcacttttcggggaaatgtgcgcggaacccctatttgtttatttttctaaatacattcaaatatgtatccgctcatgagacaataaccctgataaatgcttcaataatattgaaaaaggaagagtatgagtattcaacatttccgtgtcgcccttattcccttttttgcggcattttgccttcctgtttttgctcacccagaaacgctggtgaaagtaaaagatgctgaagatcagttgggtgcacgagtgggttacatcgaactggatctcaacagcggtaagatccttgagagttttcgccccgaagaacgttttccaatgatgagcacttttaaagttctgctatgtggcgcggtattatcccgtattgacgccgggcaagagcaactcggtcgccgcatacactattctcagaatgacttggttgagtactcaccagtcacagaaaagcatcttacggatggcatgacagtaagagaattatgcagtgctgccataaccatgagtgataacactgcggccaacttacttctgacaacgatcggaggaccgaaggagctaaccgcttttttgcacaacatgggggatcatgtaactcgccttgatcgttgggaaccggagctgaatgaagccataccaaacgacgagcgtgacaccacgatgcctgtagcaatggcaacaacgttgcgcaaactattaactggcgaactacttactctagcttcccggcaacaattaatagactggatggaggcggataaagttgcaggaccacttctgcgctcggcccttccggctggctggtttattgctgataaatctggagccggtgagcgtgggtctcgcggtatcattgcagcactggggccagatggtaagccctcccgtatcgtagttatctacacgacggggagtcaggcaactatggatgaacgaaatagacagatcgctgagataggtgcctcactgattaagcattggtaactgtcagaccaagtttactcatatatactttagattgatttaaaacttcatttttaatttaaaaggatctaggtgaagatcctttttgataatctcatgaccaaaatcccttaacgtgagttttcgttccactgagcgtcagaccccgtagaaaagatcaaaggatcttcttgagatcctttttttctgcgcgtaatctgctgcttgcaaacaaaaaaaccaccgctaccagcggtggtttgtttgccggatcaagagctaccaactctttttccgaaggtaactggcttcagcagagcgcagataccaaatactgtccttctagtgtagccgtagttaggccaccacttcaagaactctgtagcaccgcctacatacctcgctctgctaatcctgttaccagtggctgctgccagtggcgataagtcgtgtcttaccgggttggactcaagacgatagttaccggataaggcgcagcggtcgggctgaacggggggttcgtgcacacagcccagcttggagcgaacgacctacaccgaactgagatacctacagcgtgagcattgagaaagcgccacgcttcccgaagggagaaaggcggacaggtatccggtaagcggcagggtcggaacaggagagcgcacgagggagcttccagggggaaacgcctggtatctttatagtcctgtcgggtttcgccacctctgacttgagcgtcgatttttgtgatgctcgtcaggggggcggagcctatggaaaaacgccagcaacgcggcctttttacggttcctggccttttgctggccttttgctcacatgttctttcctgcgttatcccctgattctgtggataaccgtattaccgcctttgagtgagctgataccgctcgccgcagccgaacgaccgagcgcagcgagtcagtgagcgaggaagcggaagagcgcccaatacgcaaaccgcctctccccgcgcgttggccgattcattaatgcagctggcacgacaggtttcccgactggaaagcgggcagtgagcgcaacgcaattaatgtgagttagctcactcattaggcaccccaggctttacactttatgcttccggctcgtatgttgtgtggaattgtgagcggataacaatttcacacaggaaacagctatgaccatgattacgcc

SEQ ID NO: 5 - DNA, 720 bp, Artificial
  chimeric antigen receptor
gacattgtgatgacccagtctcacaaattcatgtccacatcaattggagccagggtcagcatcacctgcaaggccagtcaggatgtgagaactgctgtagcctggtatcaacagaaaccaggccagtctcctaaactactaatttactcggcatcctaccggtacactggagtccctgatcgcttcactggcagtggatctgggacggatttcactttcaccatcagcagtgtgcaggctgaagacctggcagtttattactgtcagcaacattatggtactcctccgtggacgttcggtggaggcaccaagctggaaatcaaaggcggcggaggatctggcggaggcggaagtggcggagggggctctgaagtgcagctggtggagtctgggggaggcttagtgaagcctggagggtccctgaaactctcctgtgaagcctctagattcactttcagtagctatgccatgtcttgggttcgccagactccggagaagaggctggagtgggtcgcagccattagtggaggtggtaggtacacctactatccagacagtatgaagggtcgattcaccatctccagagacaatgccaagaatttcctgtacctgcaaatgagcagtctgaggtctgaggacacggccatgtattactgtgcaagacactatgatggttatcttgactactggggccaaggcaccactctcacagtctcctca